European Patent Specification EP 4 422 622 B1, published June 18, 2025. Title: GAMMA-SECRETASE INHIBITORS FOR USE IN THE TREATMENT OF INHERITED EPIDERMOLYSIS BULLOSA. Applicant: Ospedale Pediatrico Bambino Gesù. The sequence listing filed with the application follows.

SEQUENCE LISTING (24 sequences)

SEQ ID NO: 1 - DNA, 21 bp, synthetic construct
  misc_feature 1..19: note = RNA
  misc_feature 20..21: note = DNA
  source 1..21: mol_type = other DNA
gaatgtgaggccaaacctttt

SEQ ID NO: 2 - DNA, 21 bp, synthetic construct
  misc_feature 1..19
  misc_feature 20..21: note = DNA
  source 1..21: mol_type = other DNA
cctgtaacatagcccgaaatt

SEQ ID NO: 3 - DNA, 20 bp, synthetic construct
  source 1..20: mol_type = other DNA
gcgtggctattccttcgtta

SEQ ID NO: 4 - DNA, 21 bp, synthetic construct
  source 1..21: mol_type = other DNA
gactccatcccgatgaaggat

SEQ ID NO: 5 - DNA, 20 bp, synthetic construct
  source 1..20: mol_type = other DNA
ggcccagaagtatgaccacc

SEQ ID NO: 6 - DNA, 24 bp, synthetic construct
  source 1..24: mol_type = other DNA
gatgaattcgcaaagaatgatgcc

SEQ ID NO: 7 - DNA, 20 bp, synthetic construct
  source 1..20: mol_type = other DNA
ggccaagacgaagacatccc

SEQ ID NO: 8 - DNA, 20 bp, synthetic construct
  source 1..20: mol_type = other DNA
cgtcatcgcacaacaccttg

SEQ ID NO: 9 - DNA, 19 bp, synthetic construct
  source 1..19: mol_type = other DNA
gaaggtgaaggtcggagtc

SEQ ID NO: 10 - DNA, 20 bp, synthetic construct
  source 1..20: mol_type = other DNA
gaagatggtgatgggatttc

SEQ ID NO: 11 - DNA, 21 bp, synthetic construct
  source 1..21: mol_type = other DNA
agaaagatagctcgcggcatt

SEQ ID NO: 12 - DNA, 20 bp, synthetic construct
  source 1..20: mol_type = other DNA
tacttccccagcacacttgg

SEQ ID NO: 13 - DNA, 20 bp, synthetic construct
  source 1..20: mol_type = other DNA
gtctcaacgggggaacttgt

SEQ ID NO: 14 - DNA, 20 bp, synthetic construct
  source 1..20: mol_type = other DNA
gcgtgctcagcaatttcaca

SEQ ID NO: 15 - DNA, 20 bp, synthetic construct
  source 1..20: mol_type = other DNA
gacagcctcaacgggtacaa

SEQ ID NO: 16 - DNA, 20 bp, synthetic construct
  source 1..20: mol_type = other DNA
cacacgtagccactggtcat

SEQ ID NO: 17 - DNA, 22 bp, synthetic construct
  source 1..22: mol_type = other DNA
tggaagagacggtcacttcaca

SEQ ID NO: 18 - DNA, 23 bp, synthetic construct
  source 1..23: mol_type = other DNA
gtggtacttcataagagcttcgg

SEQ ID NO: 19 - DNA, 19 bp, synthetic construct
  source 1..19: mol_type = other DNA
aactccagctggtccttag

SEQ ID NO: 20 - DNA, 19 bp, synthetic construct
  source 1..19: mol_type = other DNA
tcttgaaccctcatcctgt

SEQ ID NO: 21 - DNA, 18 bp, synthetic construct
  source 1..18: mol_type = other DNA
aaccaccggggtgagagg

SEQ ID NO: 22 - DNA, 20 bp, synthetic construct
  source 1..20: mol_type = other DNA
ggggaaagctccttggaagt

SEQ ID NO: 23 - DNA, 20 bp, synthetic construct
  source 1..20: mol_type = other DNA
tgacactggcaaaacaatgc

SEQ ID NO: 24 - DNA, 21 bp, synthetic construct
  source 1..21: mol_type = other DNA
ggtccttttcaccagcaagct